European Patent Application EP 4 725 967 A1, published April 15, 2026. Title: 结合人CCR8的抗体及其用途. Applicant: 南京蓬勃生物科技有限公司. Application CN. The sequence listing filed with the application follows.

SEQUENCE LISTING (40 sequences)

SEQ ID NO: 1 - protein, 5 aa, synthetic construct
AYAMN

SEQ ID NO: 2 - protein, 19 aa, synthetic construct
RIRSKSNYYATYYADSVKD

SEQ ID NO: 3 - protein, 15 aa, synthetic construct
QGYFGTRESRRYFDV

SEQ ID NO: 4 - protein, 11 aa, synthetic construct
KASESVGSYVS

SEQ ID NO: 5 - protein, 7 aa, synthetic construct
GASTRYT

SEQ ID NO: 6 - protein, 9 aa, synthetic construct
GQNYIYPLT

SEQ ID NO: 7 - protein, 5 aa, synthetic construct
DFEMH

SEQ ID NO: 8 - protein, 17 aa, synthetic construct
AFDPETGGTAYNQKFKG

SEQ ID NO: 9 - protein, 8 aa, synthetic construct
RLRRHFDS

SEQ ID NO: 10 - protein, 16 aa, synthetic construct
RSSQSLVHSYGNTYLH

SEQ ID NO: 11 - protein, 7 aa, synthetic construct
KVSNRFS

SEQ ID NO: 12 - protein, 9 aa, synthetic construct
SQSTHVPFT

SEQ ID NO: 13 - protein, 5 aa, synthetic construct
TYAMN

SEQ ID NO: 14 - protein, 12 aa, synthetic construct
GGNSYGSSYFDY

SEQ ID NO: 15 - protein, 16 aa, synthetic construct
RSSKSLLHRNGNTYLY

SEQ ID NO: 16 - protein, 7 aa, synthetic construct
RMSNLAS

SEQ ID NO: 17 - protein, 9 aa, synthetic construct
MQHLEYPFT

SEQ ID NO: 18 - protein, 5 aa, synthetic construct
TYAMY

SEQ ID NO: 19 - protein, 19 aa, synthetic construct
RIRSKSNNYATYYADSVKD

SEQ ID NO: 20 - protein, 12 aa, synthetic construct
GGRGNYLYAMDY

SEQ ID NO: 21 - protein, 16 aa, synthetic construct
RSSKSLLHSNGNTYLY

SEQ ID NO: 22 - protein, 126 aa, synthetic construct
EVQLVESGGGLVQPKGSLKLSCAASGFNFNAYAMNWVRQAPGKGLEWVARIRSKSNYYATYYADSVKDRFTISRDDSESMLYLQMNNLKTEDTAMYYCVRQGYFGTRESRRYFDVWGTGTTVTVSS

SEQ ID NO: 23 - protein, 107 aa, synthetic construct
NIVMTQSPKSMSMSVGERVTLSCKASESVGSYVSWYQQKPGQSPKLLIYGASTRYTGVPDRFTGSGSAKDFTLTISSVQAEDPADYHCGQNYIYPLTFGAGTKLELK

SEQ ID NO: 24 - protein, 126 aa, synthetic construct
EVQLVESGGGLVQPGGSLKLSCAASGFNFNAYAMNWVRQASGKGLEWVGRIRSKSNYYATYYADSVKDRFTISRDDSKNTAYLQMNSLKTEDTAVYYCVRQGYFGTRESRRYFDVWGQGTLVTVSS

SEQ ID NO: 25 - protein, 107 aa, synthetic construct
EIVLTQSPGTLSLSPGERATLSCKASESVGSYVSWYQQKPGQAPRLLIYGASTRYTGIPARFSGSGSGTDFTLTISSLEPEDFAVYYCGQNYIYPLTFGGGTKLEIK

SEQ ID NO: 26 - protein, 126 aa, synthetic construct
EVQLVESGGGLVQPGRSLRLSCTASGFNFNAYAMNWVRQAPGKGLEWVGRIRSKSNYYATYYADSVKDRFTISRDDSKSIAYLQMNSLKTEDTAVYYCVRQGYFGTRESRRYFDVWGQGTLVTVSS

SEQ ID NO: 27 - protein, 117 aa, synthetic construct
QVQLQQSGAELVRPGASVTLSCKTSGYTFTDFEMHWVKQTPVHGLEWIGAFDPETGGTAYNQKFKGKAILTADKSSSTAYMELRSLTSEDSAVYYCTGRLRRHFDSWGQGTTLTVSS

SEQ ID NO: 28 - protein, 112 aa, synthetic construct
DVVMTQTPLSLPVSLGDQASISCRSSQSLVHSYGNTYLHWYLQKPGQSPKLLIYKVSNRFSGVPDRFSGSGSGTDFTLKISRVEAEDLGVYFCSQSTHVPFTFGSGTKLEIK

SEQ ID NO: 29 - protein, 117 aa, synthetic construct
QVQLVQSGAEVKKPGASVKVSCKVSGYTFTDFEMHWVRQAPGKGLEWIGAFDPETGGTAYNQKFKGRVTMTEDTSTDTAYMELSSLRSEDTAVYYCTGRLRRHFDSWGQGTLVTVSS

SEQ ID NO: 30 - protein, 112 aa, synthetic construct
DIVMTQSPLSLPVTPGEPASISCRSSQSLVHSYGNTYLHWYLQKPGQSPQLLIYKVSNRFSGVPDRFSGSGSGTDFTLKISRVEAEDVGVYYCSQSTHVPFTFGQGTKLEIK

SEQ ID NO: 31 - protein, 123 aa, synthetic construct
EVQLVESGGGLVQPKGSLKLSCAASGFSFNTYAMNWVRQAPGKGLEWVARIRSKSNYYATYYADSVKDRFTISRDDSESMLYLQMNNLKTEDTAMYYCVRGGNSYGSSYFDYWGQGTTLTVSS

SEQ ID NO: 32 - protein, 112 aa, synthetic construct
DIVMTQAAPSVPVTPGESVSISCRSSKSLLHRNGNTYLYWFLQRPGQSPQLLIYRMSNLASGVPDRFSGSGSGTAFTLRISRLEAEDVGVYYCMQHLEYPFTFGAGTKLELK

SEQ ID NO: 33 - protein, 123 aa, synthetic construct
EVQLVESGGGLVKPGGSLRLSCAASGFSFNTYAMNWVRQAPGKGLEWVGRIRSKSNYYATYYADSVKDRFTISRDDSKNTLYLQMNSLKTEDTAVYYCVRGGNSYGSSYFDYWGQGTLVTVSS

SEQ ID NO: 34 - protein, 112 aa, synthetic construct
DIVMTQSPLSLPVTPGEPASISCRSSKSLLHRNGNTYLYWYLQKPGQSPQLLIYRMSNLASGVPDRFSGSGSGTDFTLKISRVEAEDVGVYYCMQHLEYPFTFGQGTKLEIK

SEQ ID NO: 35 - protein, 123 aa, synthetic construct
EVQLVESGGGLVQPKGSLKLSCAASGFTFNTYAMYWVCQAPGKGLEWVARIRSKSNNYATYYADSVKDRFTISRDDSQSMLYLQMNNLKTEDTAMYYCVRGGRGNYLYAMDYWGQGTSVTVSS

SEQ ID NO: 36 - protein, 112 aa, synthetic construct
DIVMTQAAPSVPVTPGESVSISCRSSKSLLHSNGNTYLYWFLQRPGQSPQLLIYRMSNLASGVPDRFSGSGSGSAFTLRISRVEAEDVGVYYCMQHLEYPFTFGSGTKLEIK

SEQ ID NO: 37 - protein, 330 aa, synthetic construct [sequence omitted]

SEQ ID NO: 38 - protein, 107 aa, synthetic construct [sequence omitted]

SEQ ID NO: 39 - protein, 330 aa, synthetic construct
AKTTAPSVYPLAPVCGDTTGSSVTLGCLVKGYFPEPVTLTWNSGSLSSGVHTFPAVLQSDLYTLSSSVTVTSSTWPSQSITCNVAHPASSTKVDKKIEPRGPTIKPCPPCKCPAPNLLGGPSVFIFPPKIKDVLMISLSPIVTCVVVDVSEDDPDVQISWFVNNVEVHTAQTQTHREDYNSTLRVVSALPIQHQDWMSGKEFKCKVNNKDLPAPIERTISKPKGSVRAPQVYVLPPPEEEMTKKQVTLTCMVTDFMPEDIYVEWTNNGKTELNYKNTEPVLDSDGSYFMYSKLRVEKKNWVERNSYSCSVVHEGLHNHHTTKSFSRTPGK

SEQ ID NO: 40 - protein, 107 aa, synthetic construct
RADAAPTVSIFPPSSEQLTSGGASVVCFLNNFYPKDINVKWKIDGSERQNGVLNSWTDQDSKDSTYSMSSTLTLTKDEYERHNSYTCEATHKTSTSPIVKSFNRNEC